European Patent Application EP 4 488 372 A2, published January 8, 2025. Title: METHOD FOR ENHANCING SENSITIVITY OF ENDOTOXIN MEASURING AGENT. Applicant: Seikagaku Corporation. Application EP. The sequence listing filed with the application follows.

SEQUENCE LISTING (12 sequences)

SEQ ID NO: 1 - DNA, 3060 bp, Tachypleus tridentatus
  source 1..3060: mol_type = genomic DNA
atggtcttagcgtcgtttttggtgtctggtttagttctagggatactagcccaacaaatgcgtccagttcagtccagaggagtagatctgggcttgtgtgatgaaacgaggttcgagtgtaagtgtggagatccaggctatgtgttcaacgtccctatgaaacaatgcacgtacttctatcgatggaggccttattgtaaaccatgtgatgacctggaggctaaggacatttgtccaaagtacaaacgatgtcaagagtgtaaggctggtcttgatagttgtgttacttgtccacctaacaaatatggtacttggtgtagcggtgaatgtcaatgtaagaatggaggtatctgtgaccagaggacaggagcttgtacctgtcgtgacagatatgaaggagcgcactgtgaaattctcaaaggttgtcctcttcttccatcggattctcaagttcaggaagtcagaaacccaccagataatccccaaactattgactacagctgttcaccagggttcaagcttaaaggcgtggcacgaattagctgtctcccaaatggacagtggagtagctttccacccaaatgtattcgagaatgtgccaaggtttcatctccagaacacgggaaagtgaatgctcctagtggcaatatgatagaaggggctactttacggttctcatgtgatagtccctactacttgattggtcaagaaacattaacctgccagggtaatggtcagtggagtggacaaataccacaatgtaagaagttggtcttctgtcctgaccttgatcctgtaaaccatgctgaacaccaggttaaaattggtgtggaacaaaaatatggtcagtttcctcaaggcactgaagtgacctatacgtgttcgggtaactacttcttgatgggttttaacaccttaaaatgtaaccctgatgggtcctggtcaggatcacagccatcctgtgttaaagtggcagacagagaggtcgactgtgacagtaaagctgtagacttcttggatgatgttggtgaacctgtcaggatccactgtcctgctggctgttctttgacagctggtactgtgtggggtacagccatataccacgaactttcctcagtgtgtcgtgcagccatccatgctggcaagcttccaaactctggaggggcggtgcatgtagtgaacaatggcccctactcggactttctgggtagtgacctgaatgggataaaatcggaagagttgaagtctcttgcccgcagttttcgatttgattatgtcagttcatccacagcaggtagatcaggatgtcctgatggatggtttgaggtagaagagaactgtgtgtacgttacatcaaaacagagagcctgggaaagagctcaaggtgtgtgtaccaatatggctgctcgtcttgctgtgctagacaaagatctaattccgagttccttgactgagactctacgagggaaagggttaacaaccacatggataggattgcacagactagatgctgagaagccctttgtttgggagctaatggatcgtagtaatgtggttctgaatgataacctaacattctgggcctctggcgaacctggaaatgaaactaactgtgtatatctggacatccgagatcagctgcagcctgtgtggaaaaccaagtcatgttttcagccctcaagctttgcttgcatgatggatttgtcagacagaaataaagccaaatgcgatgaccctggaccactggaaaatggacacgccacacttcatggacaaagtattgatgggttctatgctggttcttctataaggtacagctgtgaggttctccactacctcagtggaactgagaccgtaacttgtacaacaaatggcacatggagtgctcctaaacctcgatgtatcaaagtcatcacctgccaaaaccctcctgtaccatcatatggttctgtggaaatcaaacccccaagtcggacaaactcgatcagtcgtgttgggtcacctttcttgaggttgccacggttacccctcccattagccagagcagccaaacctcctccaaaacctagatcctcacaaccctctactgtggacttggcttctaaagttaaactacctgaaggtcattaccgggtagggtctcgagccatttacacgtgcgagtcgagatactacgaactacttggatctcaaggcagaagatgtgactctaatggaaactggagtggtcggcccgctagctgtattccagtttgtggacggtcagactctcctcgttctcctttcatctggaatgggaattctacagaaataggtcagtggccgtggcaggcaggaatctctcgatggcttgcagaccacaatatgtggtttctccagtgtggaggatccctattgaatgagaaatggatcgtcactgctgcccactgtgtcacctactctgctactgctgagataattgatcccagtcagtttaaaatctatctgggcaagtactaccgtgatgacagtagagacgatgactacgtacaagtaagagaggctctcgagatccacgtaaatcctaactacgaccccggcaatctcaactttgacatagccctaattcaactgaaaactcctgttactttgacaacacgagtccaaccaatctgtctgcctactgacatcacaacaagagaacacttgaaggagggaacattagcagtggtgacaggttggggtttgaatgaaaacaacacatattcagagatgattcaacaagctgtgctacctgttgttgcagcaagcacctgtgaagaggggtacaaggaagcagacttaccactgacagtaacagagaacatgttctgtgcaggttacaagaagggacgttatgatgcctgcagtggggacagtggaggaccattagtgtttgctgatgattcccgtaccgaaaggcggtgggtcttggaagggattgtcagctggggcagtcccagtggatgtggcaaggctaaccagtatgggggcttcactaaagttaacgtttttctatcatggattaggcagttcatttga

SEQ ID NO: 2 - protein, 1019 aa, Tachypleus tridentatus
MVLASFLVSGLVLGILAQQMRPVQSRGVDLGLCDETRFECKCGDPGYVFNVPMKQCTYFYRWRPYCKPCDDLEAKDICPKYKRCQECKAGLDSCVTCPPNKYGTWCSGECQCKNGGICDQRTGACTCRDRYEGAHCEILKGCPLLPSDSQVQEVRNPPDNPQTIDYSCSPGFKLKGVARISCLPNGQWSSFPPKCIRECAKVSSPEHGKVNAPSGNMIEGATLRFSCDSPYYLIGQETLTCQGNGQWSGQIPQCKKLVFCPDLDPVNHAEHQVKIGVEQKYGQFPQGTEVTYTCSGNYFLMGFNTLKCNPDGSWSGSQPSCVKVADREVDCDSKAVDFLDDVGEPVRIHCPAGCSLTAGTVWGTAIYHELSSVCRAAIHAGKLPNSGGAVHVVNNGPYSDFLGSDLNGIKSEELKSLARSFRFDYVSSSTAGRSGCPDGWFEVEENCVYVTSKQRAWERAQGVCTNMAARLAVLDKDLIPSSLTETLRGKGLTTTWIGLHRLDAEKPFVWELMDRSNVVLNDNLTFWASGEPGNETNCVYLDIRDQLQPVWKTKSCFQPSSFACMMDLSDRNKAKCDDPGPLENGHATLHGQSIDGFYAGSSIRYSCEVLHYLSGTETVTCTTNGTWSAPKPRCIKVITCQNPPVPSYGSVEIKPPSRTNSISRVGSPFLRLPRLPLPLARAAKPPPKPRSSQPSTVDLASKVKLPEGHYRVGSRAIYTCESRYYELLGSQGRRCDSNGNWSGRPASCIPVCGRSDSPRSPFIWNGNSTEIGQWPWQAGISRWLADHNMWFLQCGGSLLNEKWIVTAAHCVTYSATAEIIDPSQFKIYLGKYYRDDSRDDDYVQVREALEIHVNPNYDPGNLNFDIALIQLKTPVTLTTRVQPICLPTDITTREHLKEGTLAVVTGWGLNENNTYSEMIQQAVLPVVAASTCEEGYKEADLPLTVTENMFCAGYKKGRYDACSGDSGGPLVFADDSRTERRWVLEGIVSWGSPSGCGKANQYGGFTKVNVFLSWIRQFI

SEQ ID NO: 3 - DNA, 3060 bp, Carcinoscorpius rotundicauda
  source 1..3060: mol_type = genomic DNA
atggtcttagcgtcgtttttggtgtctggtttagttctagggctactagcccaaaaaatgcgcccagttcagtccaaaggagtagatctaggcttgtgtgatgaaacgaggttcgagtgtaagtgtggcgatccaggctatgtgttcaacattccagtgaaacaatgtacatacttttatcgatggaggccgtattgtaaaccatgtgatgacctggaggctaaggatatttgtccaaagtacaaacgatgtcaagagtgtaaggctggtcttgatagttgtgttacttgtccacctaacaaatatggtacttggtgtagcggtgaatgtcagtgtaagaatggaggtatctgtgaccagaggacaggagcttgtgcatgtcgtgacagatatgaaggggtgcactgtgaaattctcaaaggttgtcctcttcttccatcggattctcaggttcaggaagtcagaaatccaccagataatccccaaactattgactacagctgttcaccagggttcaagcttaagggtatggcacgaattagctgtctcccaaatggacagtggagtaactttccacccaaatgtattcgagaatgtgccatggtttcatctccagaacatgggaaagtgaatgctcttagtggtgatatgatagaaggggctactttacggttctcatgtgatagtccctactacttgattggtcaagaaacattaacctgtcagggtaatggtcagtggaatggacagataccacaatgtaagaacttggtcttctgtcctgacctggatcctgtaaaccatgctgaacacaaggttaaaattggtgtggaacaaaaatatggtcagtttcctcaaggcactgaagtgacctatacgtgttcgggtaactacttcttgatgggttttgacaccttaaaatgtaaccctgatgggtcttggtcaggatcacagccatcctgtgttaaagtggcagacagagaggtcgactgtgacagtaaagctgtagacttcttggatgatgttggtgaacctgtcaggatccactgtcctgctggctgttctttgacagctggtactgtgtggggtacagccatataccatgaactttcctcagtgtgtcgtgcagccatccatgctggcaagcttccaaactctggaggagcggtgcatgttgtgaacaatggcccctactcggactttctgggtagtgacctgaatgggataaaatcggaagagttgaagtctcttgcccggagtttccgattcgattatgtccgttcctccacagcaggtaaatcaggatgtcctgatggatggtttgaggtagacgagaactgtgtgtacgttacatcaaaacagagagcctgggaaagagctcaaggtgtgtgtaccaatatggctgctcgtcttgctgtgctggacaaagatgtaattccaaattcgttgactgagactctacgagggaaagggttaacaaccacgtggataggattgcacagactagatgctgagaagccctttatttgggagttaatggatcgtagtaatgtggttctgaatgataacctaacattctgggcctctggcgaacctggaaatgaaactaactgtgtatatatggacatccaagatcagttgcagtctgtgtggaaaaccaagtcatgttttcagccctcaagttttgcttgcatgatggatctgtcagacagaaataaagccaaatgcgatgatcctggatcactggaaaatggacacgccacacttcatggacaaagtattgatgggttctatgctggttcttctataaggtacagctgtgaggttctccactacctcagtggaactgaaaccgtaacttgtacaacaaatggcacatggagtgctcctaaacctcgatgtatcaaagtcatcacctgccaaaacccccctgtaccatcatatggttctgtggaaatcaaacccccaagtcggacaaactcgataagtcgtgttgggtcacctttcttgaggttgccacggttacccctcccattagctagagcagccaaacctcctccaaaacctagatcctcacaaccctctactgtggacttggcttctaaagttaaactacctgaaggtcattaccgggtagggtctcgagccatctacacgtgcgagtcgagatactacgaactacttggatctcaaggcagaagatgtgactctaatggaaactggagtggtcggccagcgagctgtattccagtttgtggacggtcagactctcctcgttctccttttatctggaatgggaattctacagaaataggtcagtggccgtggcaggcaggaatctctagatggcttgcagaccacaatatgtggtttctccagtgtggaggatctctattgaatgagaaatggatcgtcactgctgcccactgtgtcacctactctgctactgctgagattattgaccccaatcagtttaaaatgtatctgggcaagtactaccgtgatgacagtagagacgatgactatgtacaagtaagagaggctcttgagatccacgtgaatcctaactacgaccccggcaatctcaactttgacatagccctaattcaactgaaaactcctgttactttgacaacacgagtccaaccaatctgtctgcctactgacatcacaacaagagaacacttgaaggagggaacattagcagtggtgacaggttggggtttgaatgaaaacaacacctattcagagacgattcaacaagctgtgctacctgttgttgcagccagcacctgtgaagaggggtacaaggaagcagacttaccactgacagtaacagagaacatgttctgtgcaggttacaagaagggacgttatgatgcctgcagtggggacagtggaggacctttagtgtttgctgatgattcccgtaccgaaaggcggtgggtcttggaagggattgtcagctggggcagtcccagtggatgtggcaaggcgaaccagtacgggggcttcactaaagttaacgttttcctgtcatggattaggcagttcatttga

SEQ ID NO: 4 - protein, 1019 aa, Carcinoscorpius rotundicauda
MVLASFLVSGLVLGLLAQKMRPVQSKGVDLGLCDETRFECKCGDPGYVFNIPVKQCTYFYRWRPYCKPCDDLEAKDICPKYKRCQECKAGLDSCVTCPPNKYGTWCSGECQCKNGGICDQRTGACACRDRYEGVHCEILKGCPLLPSDSQVQEVRNPPDNPQTIDYSCSPGFKLKGMARISCLPNGQWSNFPPKCIRECAMVSSPEHGKVNALSGDMIEGATLRFSCDSPYYLIGQETLTCQGNGQWNGQIPQCKNLVFCPDLDPVNHAEHKVKIGVEQKYGQFPQGTEVTYTCSGNYFLMGFDTLKCNPDGSWSGSQPSCVKVADREVDCDSKAVDFLDDVGEPVRIHCPAGCSLTAGTVWGTAIYHELSSVCRAAIHAGKLPNSGGAVHVVNNGPYSDFLGSDLNGIKSEELKSLARSFRFDYVRSSTAGKSGCPDGWFEVDENCVYVTSKQRAWERAQGVCTNMAARLAVLDKDVIPNSLTETLRGKGLTTTWIGLHRLDAEKPFIWELMDRSNVVLNDNLTFWASGEPGNETNCVYMDIQDQLQSVWKTKSCFQPSSFACMMDLSDRNKAKCDDPGSLENGHATLHGQSIDGFYAGSSIRYSCEVLHYLSGTETVTCTTNGTWSAPKPRCIKVITCQNPPVPSYGSVEIKPPSRTNSISRVGSPFLRLPRLPLPLARAAKPPPKPRSSQPSTVDLASKVKLPEGHYRVGSRAIYTCESRYYELLGSQGRRCDSNGNWSGRPASCIPVCGRSDSPRSPFIWNGNSTEIGQWPWQAGISRWLADHNMWFLQCGGSLLNEKWIVTAAHCVTYSATAEIIDPNQFKMYLGKYYRDDSRDDDYVQVREALEIHVNPNYDPGNLNFDIALIQLKTPVTLTTRVQPICLPTDITTREHLKEGTLAVVTGWGLNENNTYSETIQQAVLPVVAASTCEEGYKEADLPLTVTENMFCAGYKKGRYDACSGDSGGPLVFADDSRTERRWVLEGIVSWGSPSGCGKANQYGGFTKVNVFLSWIRQFI

SEQ ID NO: 5 - DNA, 1203 bp, Tachypleus tridentatus
  source 1..1203: mol_type = genomic DNA
atgacgtggatatgtgtgataacgttgtttgctctggcttctgctacgttgggtaacaaagttagtagagtgggggtcctcttccccaagacacggaacgacaatgagtgtacagcaagagggggattgaaaggatcctgcaaatccctcatagactgtcctagtgtcttggctacgttgaaggacagttttcctgtcgtttgctcttggaatggtcgatttcagcctattgtctgctgtcctgatgcaatagcaccaccacctgtaaccacaacagctgtaactgtaatatctacaaaagaaccaaagcttccaagattacatatatcaggttgtggaaaaagaaaagtcaaaatagatattacaactgttggacgctctggatcaccaatacttcctccgatatctactcctcaaaattcaacaggtgggagaggaattattgctggaggcgtagaagccaaaattggcgcgtggccttggatggcagctgtttttgtgaaaaactttggcattggcagattccactgtgctggtagcataatcagtaacaagtacattttgtcagctgcccacgccttccttatcggaggtcgaaagttgaccccaactcgcttagctgtccgtgtgggaggccactacataaagaggggtcaagagtatccagtgaaagacgtgattatccatcctcattatgtagaaaaggagaactacaatgatatagccataatcgagttaaaagaggaactgaactttacggacttggtcaatcctatatgtctccctgatccagagacagtaacggatccattaaaagacagaattgtgactgcagcgggatggggcgatctggatttctccggtccacggagccaagttctacgtgaggtaagcatcccagttgttccagttgataaatgtgatcaagcctatgagaaactcaacaccccttcactaaaaaatgggataacgaataacttcctttgcgctggattggaagaaggagggaaagacgcttgccaaggcgattctggtggaccgttgatgctagtgaacaacactaggtggatagtagtaggagttgtgtcgttcgggcacaagtgtgccgaggaaggatatcctggtgtgtactcgcgcgtagcgagttacctagactggatcgcgaaagttacgaactcgttagatcatgccgtcactaactaa

SEQ ID NO: 6 - protein, 400 aa, Tachypleus tridentatus
MTWICVITLFALASATLGNKVSRVGVLFPKTRNDNECTARGGLKGSCKSLIDCPSVLATLKDSFPVVCSWNGRFQPIVCCPDAIAPPPVTTTAVTVISTKEPKLPRLHISGCGKRKVKIDITTVGRSGSPILPPISTPQNSTGGRGIIAGGVEAKIGAWPWMAAVFVKNFGIGRFHCAGSIISNKYILSAAHAFLIGGRKLTPTRLAVRVGGHYIKRGQEYPVKDVIIHPHYVEKENYNDIAIIELKEELNFTDLVNPICLPDPETVTDPLKDRIVTAAGWGDLDFSGPRSQVLREVSIPVVPVDKCDQAYEKLNTPSLKNGITNNFLCAGLEEGGKDACQGDSGGPLMLVNNTRWIVVGVVSFGHKCAEEGYPGVYSRVASYLDWIAKVTNSLDHAVTN

SEQ ID NO: 7 - DNA, 1128 bp, Tachypleus tridentatus
  source 1..1128: mol_type = genomic DNA
atgttggtgaataacgtgttttcactactgtgtttcccactcttgatgtctgtggttagatgcagtactctcagcagacagcgtagacagtttgttttccctgacgaggaagaactttgctcaaaccgatttactgaagaaggaacatgcaaaaatgtcttggattgtagaatacttttacaaaaaaatgattataatttactcaaagaatcaatatgcggctttgaaggcataacacccaaagtttgttgtccgaaatcaagccatgtaatttcaagtacacaggcacctccagaaaccactacgactgaacgcccaccaaaacagataccacccaatcttcctgaagtgtgtggaattcacaatactacaactaccaggattattggaggtcgggaagcacctattggagcctggccgtggatgactgctgtctacataaaacaaggaggaatcagaagtgttcagtgtggtggcgcacttgtcactaacaggcacgtgattacagcttcgcactgtgttgtaaacagtgcaggaacagatgtgatgccagctgatgtattctcggttcgtctgggtgaacacaatttatacagtaccgatgacgattcgaatccaatagattttgcagttacgtcggtgaaacatcacgaacactttgtactcgcgacgtatttgaatgacatcgcaattctaacgttaaatgacacagttacgtttacagacagaattcgacccatttgtctaccttatcgtaagttgagatacgatgatctagcaatgagaaaaccgtttatcactggatggggaacaacagcatttaacggcccatctagtgcagtgttgagagaagtacagttaccaatatgggaacacgaggcctgtagacaggcctacgagaaggatttaaatattacaaacgtgtatatgtgtgctggctttgcagatggcgggaaggatgcttgccagggtgattctggaggtccaatgatgttgcctgttaaaaccggagagttttatctcattggaattgtgtctttcggaaagaaatgcgcattgcctggatttcctggggtttacacaaaagtgacagagtttttagattggattgcagaacatatggtgtag

SEQ ID NO: 8 - protein, 375 aa, Tachypleus tridentatus
MLVNNVFSLLCFPLLMSVVRCSTLSRQRRQFVFPDEEELCSNRFTEEGTCKNVLDCRILLQKNDYNLLKESICGFEGITPKVCCPKSSHVISSTQAPPETTTTERPPKQIPPNLPEVCGIHNTTTTRIIGGREAPIGAWPWMTAVYIKQGGIRSVQCGGALVTNRHVITASHCVVNSAGTDVMPADVFSVRLGEHNLYSTDDDSNPIDFAVTSVKHHEHFVLATYLNDIAILTLNDTVTFTDRIRPICLPYRKLRYDDLAMRKPFITGWGTTAFNGPSSAVLREVQLPIWEHEACRQAYEKDLNITNVYMCAGFADGGKDACQGDSGGPMMLPVKTGEFYLIGIVSFGKKCALPGFPGVYTKVTEFLDWIAEHMV

SEQ ID NO: 9 - DNA, 1203 bp, Tachypleus tridentatus
  source 1..1203: mol_type = other DNA
atgacctggatctgcgtgatcaccctgttcgctctggcttccgctaccctgggcaacaaggtgtcccgtgtgggtgtcctgttccccaagacccgtaacgacaacgagtgcaccgctcgtggtggtctgaagggctcctgcaagtccctgatcgactgcccctccgtgctggctaccctgaaggactccttccccgtcgtgtgctcctggaacggtcgtttccagcccatcgtgtgctgccccgacgctatcgctcccccccctgtgaccaccaccgctgtgaccgtgatctccaccaaggagcccaagctgccccgtctgcacatctccggttgcggcaagcgcaaggtcaagatcgacatcaccaccgtgggccgttccggttcccccatcctgccccccatctccaccccccagaactccactggtggtcgtggtatcatcgctggcggtgtcgaggctaagatcggtgcttggccctggatggctgctgtgttcgtgaagaacttcggtatcggtcgcttccactgcgctggttccatcatctccaacaagtacatcctgtccgctgctcacgctttcctcatcggtggtcgcaagctgacccccacccgtctggctgtgcgtgtgggtggtcactacatcaagcgtggccaggagtaccccgtcaaggacgtgatcatccacccccactacgtggagaaggagaactacaacgacatcgccatcatcgagctgaaggaggagctgaacttcaccgacctggtcaaccccatctgcctgcccgaccccgagactgtgaccgaccctctgaaggaccgtatcgtgaccgctgctggctggggcgacctggacttctccggtccccgttcccaggtgctgcgtgaggtgtccatccccgtggtgcccgtggacaagtgcgaccaggcttacgagaagctgaacaccccctccctgaagaacggtattaccaacaacttcctctgcgccggactcgaggagggtggcaaggacgcttgccagggcgactccggtggtcccctgatgctggtcaacaacacccgttggatcgtcgtgggtgtcgtgtccttcggtcacaagtgcgctgaggagggttaccccggcgtctactcccgtgtggcttcctacctggactggatcgctaaggtcaccaactccctggaccacgctgtcaccaactaa

SEQ ID NO: 10 - DNA, 3063 bp, Limulus polyphemus
  source 1..3063: mol_type = genomic DNA
atggtactagcgtcgttcttggtgtctggtttagttctagggctattagcccaacaaatgcacccagttcagtccagaggagtagatctgggcttgtgtgatgacacgaggtttgagtgtaagtgtggagatccaggatacgtgttcaacgtccccgcgaagcaatgtacgtacttctatcgatggaggccttattgtaaaccatgtgacaaactggaggctaaagatgtgtgtcccaagtacaaacgatgtcaagagtgtagggctggtctcgacagttgtgtgagttgtccacctaacaaatatggaacttggtgtagcggtgagtgtcagtgtaagaatgggggtatttgtgatcagaggacaggagcttgtacatgtcgtgacagatatgaaggtgtgcattgtgaaatccttcaaggttgtcctcttcttcaatcggatccccaggttcaggaagtaaaaaatccaccaaatgatccacaaactattgactacagctgttcaccaggcttcaagcttaaaggcgtggcacgtatcacctgtcttccaaatgggcagtggagtagctttccacccaaatgtattcgagaatgttccatggtttcatctctagaacatggcaaagtaaactctcctagtgccgatctgatagaaggagctactttaaggttctcatgtgatagtccctactacttgattggtcaagaaacattaacctgccagggcaacggtcagtggagtgggcagataccacagtgtcagaaattggtcttctgccctgaccttgaccctgtaagccatgctgaacaccaggttaaaattggcctagaacaaaaatatggtcaatttcctcaaggcactgaagtaacctatacgtgtactggtaattacttcttgatgggtttggacaccttaaaatgtaaccctgatgggtcctggtcgggaacacagccgtcctgtgttaaagtggcagacagagaggtcaactgtgacagtaaagctgtggacttcttggatgatgttggcgaacctgtcaggatccactgtcctgctggctgttccttaactgctggtactgtatggggtacagccatatatcacgaactttcctcagtatgtcgtgcagctattcatgctggcaaggttccaaactctggaggtgcagtgcatgtagtgaacaacggtccgtactcagactttctggctagtgatctgaatgggataaaatcagacgagttgaagtctcttgctcagagtttccgattcgattatgtcagttcatcaacagcagggagaaagtcaggatgtcctgatggatggttcgagattgaggagaactgtgtgtacgttacatcgaaacagagagcctgggaaagagctcaaggtgtatgtaccaatatggccgctcgtcttgctgtgttagacaaagatgtaattccaagttccttgactgagactctacgagggaaagggttagcaacgacgtggattggactacacagattagatgctgataatcactttatttgggagctaatggatcgcagtagtgttgctttgaatgacagcctaacattctgggctcctggagaacctgggaatgaaactaactgtgtatatctggatatccaagatcagctacagccagtgtggaaaaccaagtcttgttttcaaccctcaagttttgtttgtatgatggatttgtcagacaagaacaaagccaaatgcaaagaccctggacctttggaaaacggacacgccaagcttcatggtcaaagtattgatggattttatgctgggtcttctgtaagatacagctgcgaggtcctccactacctcagtggaactgagacagtatcttgtacatcaaatggcacgtggagtgcccctaaacctcgatgtattaaagtcatcacctgccaaacccctcctgtaccatcctatggttctgtggacatcaaacccccaagtagaacaaactcaatcagtcgtgttgggtcgccattcttgaggttgccacggttacccctccctttagccagagcagccggacctcctccaaaacctagatccgcaccaccctctactgtggacctgtcttccaaggtcaaactgcctgaaggtcattaccgggtggggtctcaagccatttacacgtgcgagtcaagatactacgaactgcttggatctcaaggtagaagatgcgactctaatggaaagtggagtggtcgaccagcaagctgtataccagtttgtggacggtcagactctccccgttctcctttcatcgtcaatggaaattccaccgaaataggtcagtggccgtggcaggcaggaatctccagatggcttgcagatcataatatgtggtttcttcagtgtggaggagctctactgaatgagaaatggatcattactgcagcccactgtgtcacctactctgctactgccgagatcattgacccaagtcagtttaaattctacctgggcaaatactatcgagatgacagtaaggatgatgactacgtacaagtaagagaggctatcgagatccatgtgaatcctaactacgatcctggaaatctcaactttgacatagccctgattcaactgaagacttctgttgctctgaccacacgagtgcaaccaatatgtctgcctactgatctcactacaagagaaaacctgaaagagggagcgttagcggtggtgacaggatggggtttgaatgaaaacaacacatattcagagatgattcagcaagccgttctgcctgttgttgcagcaagcacctgtgaacaaggatatcaggactcgggcttgccactgacagtgacagagaacatgttctgtgcaggttacaagcaggggcgctatgatgcctgcagtggagacagtggaggaccattagtgtttgctgatgattcccgcaccgataggcggtgggtcctggaagggatcgtcagctggggcagccccaatggatgtggcaagtctaaccagtatgggggcttcactaaagttaacgtttttctatcgtggattcggcagttcatttga

SEQ ID NO: 11 - DNA, 3063 bp, Limulus polyphemus
  source 1..3063: mol_type = other DNA
atggtgctggccagcttcctggtgtctgggctggtgctggggcttctggcccagcagatgcaccctgttcaatccagaggggttgaccttggcctgtgcgatgatacccgctttgaatgtaagtgcggggatcccgggtacgtctttaacgtgcccgctaagcaatgcacatacttctaccggtggcggccatattgcaaaccttgcgacaagcttgaggcaaaagacgtatgtcccaagtataaacgatgtcaggagtgtcgggctggcctggatagctgtgtgtcctgcccacctaacaagtacggaacctggtgttcaggcgagtgccagtgcaagaacggtggaatttgtgatcagcgtacaggtgcctgtacatgtcgtgacagatacgaaggagtgcactgcgagattctgcagggctgccccttgctccagtctgacccacaggtgcaggaagtcaagaatcctcccaacgatcctcagacgattgactattcctgctcacccggttttaagctcaagggcgtggcccgaattacttgtctccccaatggtcagtggtccagctttcctcccaagtgcattagagaatgtagcatggtgtccagtttggagcatggtaaggtcaacagtccttcagctgacctcattgagggcgcaacactccggttttcctgtgactctccctattacttgattggacaggaaaccttgacttgtcagggtaatggccaatggagtggtcagatcccacagtgccagaaactggtcttttgccccgacctggatcccgtcagccatgccgaacaccaagtgaaaatcgggctcgagcaaaagtatgggcagtttccacagggcaccgaggtgacctacacgtgtactggcaattactttctgatgggactggataccctcaaatgcaatcccgacggaagttggagtggtacacagccatcttgtgttaaagtcgcagatagggaagtaaattgcgattccaaggcagtagactttctggatgacgttggggaacctgttcgcatccattgtccagctggttgttccttgactgctggtaccgtgtggggcacagctatctatcacgagttgtcctcagtctgtagagctgccatacacgctggcaaggtccctaactctggaggcgccgtccatgtcgtgaataacggtccatactctgactttctggcctccgaccttaacggaatcaagtcagacgagcttaaatccttggcacagtctttccgcttcgactatgtgagctcttctaccgcaggacgtaagagcggctgtcccgacggctggttcgagatcgaagagaactgcgtgtacgtgacttctaagcagagggcttgggagcgagcacagggagtatgcacaaacatggccgccaggctcgctgtgctggataaggacgtcatccccagtagcctgacagaaacactgagaggcaaagggctcgccacaacttggattggactgcatcgcttggacgcagataaccactttatctgggagcttatggatcgcagctccgtggctttgaacgattctttgaccttttgggcacccggggagccaggcaatgagactaattgcgtctacctggacatacaggatcagctgcaacccgtgtggaaaacgaaatcttgcttccaaccctcctcctttgtgtgcatgatggatctgagcgacaagaacaaagccaagtgcaaagatcccggacctctggagaatgggcatgcaaagctccatggacagtcaattgatgggttctatgccggcagttccgtccgttactcctgcgaagtgctccactacctgagtgggaccgaaactgtgtcatgcacatccaatggcacctggagtgctcccaaacctagatgtattaaggtcatcacttgccaaactccacccgtgcccagctacggatctgttgacatcaagcctcctagtaggacaaacagcataagccgagtgggatcacccttcctcagactgcccagacttcctctgcctctggcccgcgctgccggacctccaccaaagccacgtagtgcacctccctctaccgttgacctgtcctcaaaagtgaagctgccagaaggccattaccgcgtcgggtcacaagccatctatacgtgtgaaagtcgctactatgagctgctgggcagccaaggcaggcggtgtgactccaatggaaagtggagcggacgaccagcctcatgcattccagtctgtggcaggagcgattccccacggagtccattcatcgtcaatggcaattctacagagattggtcagtggccttggcaggctggtatctctcggtggttggccgaccacaacatgtggtttctccagtgtggcggcgctctcctgaacgagaaatggattatcacagcagctcactgcgtaacctatagcgcaaccgccgagataatcgatccatcacagttcaagttttacctgggaaagtactacagggacgatagtaaagatgacgactacgtgcaagtgagagaggccatcgagatccacgttaaccccaactatgatcctgggaatctgaatttcgatattgccctgatccagcttaaaaccagcgttgctctgactacacgagtgcagcccatatgtctcccaactgacctgaccaccagggagaacctgaaggaaggggcccttgctgttgttaccggttggggtctgaatgagaataacacttactctgaaatgatccaacaggcagtgctgcctgtggtagctgcctctacgtgcgaacagggatatcaggactcaggacttcctctgacagtaaccgaaaacatgttctgcgccgggtataaacagggccgctatgacgcctgttccggggattccggcgggcctctggttttcgccgatgacagccggactgatcggcgatgggtgcttgagggtatcgtatcctggggctctcccaacggatgcggtaagagcaatcagtatggtggcttcaccaaagtgaacgttttcctgtcctggataaggcagttcatctga

SEQ ID NO: 12 - protein, 1020 aa, Limulus polyphemus
MVLASFLVSGLVLGLLAQQMHPVQSRGVDLGLCDDTRFECKCGDPGYVFNVPAKQCTYFYRWRPYCKPCDKLEAKDVCPKYKRCQECRAGLDSCVSCPPNKYGTWCSGECQCKNGGICDQRTGACTCRDRYEGVHCEILQGCPLLQSDPQVQEVKNPPNDPQTIDYSCSPGFKLKGVARITCLPNGQWSSFPPKCIRECSMVSSLEHGKVNSPSADLIEGATLRFSCDSPYYLIGQETLTCQGNGQWSGQIPQCQKLVFCPDLDPVSHAEHQVKIGLEQKYGQFPQGTEVTYTCTGNYFLMGLDTLKCNPDGSWSGTQPSCVKVADREVNCDSKAVDFLDDVGEPVRIHCPAGCSLTAGTVWGTAIYHELSSVCRAAIHAGKVPNSGGAVHVVNNGPYSDFLASDLNGIKSDELKSLAQSFRFDYVSSSTAGRKSGCPDGWFEIEENCVYVTSKQRAWERAQGVCTNMAARLAVLDKDVIPSSLTETLRGKGLATTWIGLHRLDADNHFIWELMDRSSVALNDSLTFWAPGEPGNETNCVYLDIQDQLQPVWKTKSCFQPSSFVCMMDLSDKNKAKCKDPGPLENGHAKLHGQSIDGFYAGSSVRYSCEVLHYLSGTETVSCTSNGTWSAPKPRCIKVITCQTPPVPSYGSVDIKPPSRTNSISRVGSPFLRLPRLPLPLARAAGPPPKPRSAPPSTVDLSSKVKLPEGHYRVGSQAIYTCESRYYELLGSQGRRCDSNGKWSGRPASCIPVCGRSDSPRSPFIVNGNSTEIGQWPWQAGISRWLADHNMWFLQCGGALLNEKWIITAAHCVTYSATAEIIDPSQFKFYLGKYYRDDSKDDDYVQVREAIEIHVNPNYDPGNLNFDIALIQLKTSVALTTRVQPICLPTDLTTRENLKEGALAVVTGWGLNENNTYSEMIQQAVLPVVAASTCEQGYQDSGLPLTVTENMFCAGYKQGRYDACSGDSGGPLVFADDSRTDRRWVLEGIVSWGSPNGCGKSNQYGGFTKVNVFLSWIRQFI